European Patent Application EP 4 796 557 A1, published August 26, 2026. Title: POLYPEPTIDE, BIOACTIVE CONJUGATE, AND PREPARATION METHOD THEREFOR AND USE THEREOF. Applicant: Unovel (ShangHai) Biopharma Co.,Ltd. Application CN. The sequence listing filed with the application follows.

SEQUENCE LISTING (68 sequences)

SEQ ID NO: 1 - protein, 7 aa, synthetic construct
  source 1..7: note = 1-P2
  SITE 7: note = X is Cit
HVLNLVX

SEQ ID NO: 2 - protein, 7 aa, synthetic construct
  source 1..7: note = 1-P3
  SITE 7: note = X is Cit
VPLSLVX

SEQ ID NO: 3 - protein, 7 aa, synthetic construct
  source 1..7: note = 1-P4
  SITE 7: note = X is Cit
IPVSLVX

SEQ ID NO: 4 - protein, 7 aa, synthetic construct
  source 1..7: note = 1-P5
  SITE 7: note = X is Cit
GPLSLVX

SEQ ID NO: 5 - protein, 7 aa, synthetic construct
  source 1..7: note = 1-P6
  SITE 7: note = X is Cit
GPASLVX

SEQ ID NO: 6 - protein, 7 aa, synthetic construct
  source 1..7: note = 1-P7
  SITE 7: note = X is Cit
GPAGLVX

SEQ ID NO: 7 - protein, 7 aa, synthetic construct
  source 1..7: note = 1-P8
  SITE 7: note = X is Cit
GPQGLVX

SEQ ID NO: 8 - protein, 7 aa, synthetic construct
  source 1..7: note = 1-P9
  SITE 7: note = X is Cit
GPLGLVX

SEQ ID NO: 9 - protein, 7 aa, synthetic construct
  source 1..7: note = 1-P10
  SITE 7: note = X is Cit
GPSGLVX

SEQ ID NO: 10 - protein, 7 aa, synthetic construct
  source 1..7: note = 1-P11
  SITE 7: note = X is Cit
GPRGLVX

SEQ ID NO: 11 - protein, 7 aa, synthetic construct
  source 1..7: note = 1-P12
  SITE 7: note = X is Cit
GPAALVX

SEQ ID NO: 12 - protein, 7 aa, synthetic construct
  source 1..7: note = 1-P13
  SITE 7: note = X is Cit
GPSALVX

SEQ ID NO: 13 - protein, 9 aa, synthetic construct
  source 1..9: note = 1-P14
HVLNLGGFG

SEQ ID NO: 14 - protein, 9 aa, synthetic construct
  source 1..9: note = 1-P15
VPLSLGGFG

SEQ ID NO: 15 - protein, 9 aa, synthetic construct
  source 1..9: note = 1-P16
IPVSLGGFG

SEQ ID NO: 16 - protein, 9 aa, synthetic construct
  source 1..9: note = 1-P17
GPLSLGGFG

SEQ ID NO: 17 - protein, 9 aa, synthetic construct
  source 1..9: note = 1-P18
GPASLGGFG

SEQ ID NO: 18 - protein, 9 aa, synthetic construct
  source 1..9: note = 1-P19
GPAGLGGFG

SEQ ID NO: 19 - protein, 9 aa, synthetic construct
  source 1..9: note = 1-P20
GPQGLGGFG

SEQ ID NO: 20 - protein, 9 aa, synthetic construct
  source 1..9: note = 1-P21
GPLGLGGFG

SEQ ID NO: 21 - protein, 9 aa, synthetic construct
  source 1..9: note = 1-P22
GPSGLGGFG

SEQ ID NO: 22 - protein, 9 aa, synthetic construct
  source 1..9: note = 1-P23
GPRGLGGFG

SEQ ID NO: 23 - protein, 9 aa, synthetic construct
  source 1..9: note = 1-P24
GPAALGGFG

SEQ ID NO: 24 - protein, 9 aa, synthetic construct
  source 1..9: note = 1-P25
GPSALGGFG

SEQ ID NO: 25 - protein, 6 aa, synthetic construct
  source 1..6: note = 2-P1
  SITE 6: note = X is Cit
PRGLVX

SEQ ID NO: 26 - protein, 6 aa, synthetic construct
  source 1..6: note = 2-P2
  SITE 6: note = X is Cit
PRSLVX

SEQ ID NO: 27 - protein, 6 aa, synthetic construct
  source 1..6: note = 2-P3
  SITE 6: note = X is Cit
PRNLVX

SEQ ID NO: 28 - protein, 6 aa, synthetic construct
  source 1..6: note = 2-P4
  SITE 6: note = X is Cit
PRPLVX

SEQ ID NO: 29 - protein, 6 aa, synthetic construct
  source 1..6: note = 2-P5
  SITE 6: note = X is Cit
  SITE 2: note = X is Cit
PXGLVX

SEQ ID NO: 30 - protein, 6 aa, synthetic construct
  source 1..6: note = 2-P6
  SITE 6: note = X is Cit
  SITE 2: note = X is Cit
PXPLVX

SEQ ID NO: 31 - protein, 7 aa, synthetic construct
  source 1..7: note = 2-P7
  SITE 7: note = X is Cit
GPRSLVX

SEQ ID NO: 32 - protein, 7 aa, synthetic construct
  source 1..7: note = 2-P8
  SITE 7: note = X is Cit
GPRPLVX

SEQ ID NO: 33 - protein, 7 aa, synthetic construct
  source 1..7: note = 2-P9
  SITE 7: note = X is Cit
GPRNLVX

SEQ ID NO: 34 - protein, 7 aa, synthetic construct
  source 1..7: note = 2-P10
  SITE 7: note = X is Cit
  SITE 2: note = X is Cit
GPXGLVX

SEQ ID NO: 35 - protein, 7 aa, synthetic construct
  source 1..7: note = 2-P11
  SITE 7: note = X is Cit
  SITE 2: note = X is Cit
GPXPLVX

SEQ ID NO: 36 - protein, 7 aa, synthetic construct
  source 1..7: note = 2-P12
  SITE 7: note = X is Cit
HPRGLVX

SEQ ID NO: 37 - protein, 7 aa, synthetic construct
  source 1..7: note = 2-P13
  SITE 7: note = X is Cit
HPRSLVX

SEQ ID NO: 38 - protein, 7 aa, synthetic construct
  source 1..7: note = 2-P14
  SITE 7: note = X is Cit
HPRPLVX

SEQ ID NO: 39 - protein, 7 aa, synthetic construct
  source 1..7: note = 2-P15
  SITE 7: note = X is Cit
HPRNLVX

SEQ ID NO: 40 - protein, 7 aa, synthetic construct
  source 1..7: note = 2-P16
  SITE 7: note = X is Cit
  SITE 3: note = X is Cit
HPXGLVX

SEQ ID NO: 41 - protein, 7 aa, synthetic construct
  source 1..7: note = 2-P17
  SITE 7: note = X is Cit
  SITE 3: note = X is Cit
HPXPLVX

SEQ ID NO: 42 - protein, 7 aa, synthetic construct
  source 1..7: note = 2-P18
  SITE 7: note = X is Cit
SPRGLVX

SEQ ID NO: 43 - protein, 7 aa, synthetic construct
  source 1..7: note = 2-P19
  SITE 7: note = X is Cit
SPRSLVX

SEQ ID NO: 44 - protein, 7 aa, synthetic construct
  source 1..7: note = 2-P20
  SITE 7: note = X is Cit
SPRPLVX

SEQ ID NO: 45 - protein, 7 aa, synthetic construct
  source 1..7: note = 2-P21
  SITE 7: note = X is Cit
SPRNLVX

SEQ ID NO: 46 - protein, 7 aa, synthetic construct
  source 1..7: note = 2-P22
  SITE 7: note = X is Cit
  SITE 2: note = X is Cit
SPXGLVX

SEQ ID NO: 47 - protein, 7 aa, synthetic construct
  source 1..7: note = 2-P23
  SITE 7: note = X is Cit
  SITE 3: note = X is Cit
SPXSLVX

SEQ ID NO: 48 - protein, 7 aa, synthetic construct
  source 1..7: note = 2-P24
  SITE 7: note = X is Cit
  SITE 3: note = X is Cit
SPXPLVX

SEQ ID NO: 49 - protein, 7 aa, synthetic construct
  source 1..7: note = 2-P25
  SITE 7: note = X is Cit
GPAPLVX

SEQ ID NO: 50 - protein, 7 aa, synthetic construct
  source 1..7: note = 2-P26
  SITE 7: note = X is Cit
GPANLVX

SEQ ID NO: 51 - protein, 7 aa, synthetic construct
  source 1..7: note = 2-P27
  SITE 7: note = X is Cit
  SITE 5: note = X is Dap(Me2)
GPRGXVX

SEQ ID NO: 52 - protein, 118 aa, synthetic construct
  source 1..118: note = h1849-H2L1 VH
EVQLVESGGGVVQPGRSLRLSCAASGFTFSDYNMAWIRQAPGKGLEWVAAIIYDGTRTYYRDSVKGRFTISRDNSKSTLYLQMDSLRAEDTAVYYCATGDSYTNFAYWGQGTLVTVSS

SEQ ID NO: 53 - protein, 106 aa, synthetic construct
  source 1..106: note = h1849-H2L1 VL
EIVLTQSPTFLSASVGDRVTITCRASSSLSYMHWYQQKPGTSPKLLIYETSKLQSGVPSRFSGSGSGTSFTLTIDSLQPEDFATYYCQQGNSYPRTFGGGTKVEIK

SEQ ID NO: 54 - protein, 118 aa, synthetic construct
  source 1..118: note = h1849-H3L3 VH
EVQLVESGGGVVQPGRSLRLSCAASGFTFSDYNMAWIRQAPGKGLEWVAAIIYDGTRTYYRDSVKGRFTISRDNSKSTLYLQMNSLRAEDTAVYYCATGDSYTNFAYWGQGTLVTVSS

SEQ ID NO: 55 - protein, 106 aa, synthetic construct
  source 1..106: note = h1849-H3L3 VL
EIVLTQSPTSLSASVGDRVTITCRASSSLSYMHWYQQKPGTSPKLLIYETSKLESGVPSRFSGSGSGTDFTLTIDSLQPEDFATYYCQQGNSYPRTFGGGTKVEIK

SEQ ID NO: 56 - protein, 213 aa, synthetic construct
  source 1..213: note = h1849-H2L1 LC
EIVLTQSPTFLSASVGDRVTITCRASSSLSYMHWYQQKPGTSPKLLIYETSKLQSGVPSRFSGSGSGTSFTLTIDSLQPEDFATYYCQQGNSYPRTFGGGTKVEIKRTVAAPSVFIFPPSDEQLKSGTASVVCLLNNFYPREAKVQWKVDNALQSGNSQESVTEQDSKDSTYSLSSTLTLSKADYEKHKVYACEVTHQGLSSPVTKSFNRGEC

SEQ ID NO: 57 - protein, 448 aa, synthetic construct
  source 1..448: note = h1849-H2L1 HC
EVQLVESGGGVVQPGRSLRLSCAASGFTFSDYNMAWIRQAPGKGLEWVAAIIYDGTRTYYRDSVKGRFTISRDNSKSTLYLQMDSLRAEDTAVYYCATGDSYTNFAYWGQGTLVTVSSASTKGPSVFPLAPSSKSTSGGTAALGCLVKDYFPEPVTVSWNSGALTSGVHTFPAVLQSSGLYSLSSVVTVPSSSLGTQTYICNVNHKPSNTKVDKKVEPKSCDKTHTCPPCPAPELLGGPSVFLFPPKPKDTLMISRTPEVTCVVVDVSHEDPEVKFNWYVDGVEVHNAKTKPREEQYNSTYRVVSVLTVLHQDWLNGKEYKCKVSNKALPAPIEKTISKAKGQPREPQVYTLPPSRDELTKNQVSLTCLVKGFYPSDIAVEWESNGQPENNYKTTPPVLDSDGSFFLYSKLTVDKSRWQQGNVFSCSVMHEALHNHYTQKSLSLSPGK

SEQ ID NO: 58 - protein, 213 aa, synthetic construct
  source 1..213: note = h1849-H3L3 LC
EIVLTQSPTSLSASVGDRVTITCRASSSLSYMHWYQQKPGTSPKLLIYETSKLESGVPSRFSGSGSGTDFTLTIDSLQPEDFATYYCQQGNSYPRTFGGGTKVEIKRTVAAPSVFIFPPSDEQLKSGTASVVCLLNNFYPREAKVQWKVDNALQSGNSQESVTEQDSKDSTYSLSSTLTLSKADYEKHKVYACEVTHQGLSSPVTKSFNRGEC

SEQ ID NO: 59 - protein, 448 aa, synthetic construct
  source 1..448: note = h1849-H3L3 HC
EVQLVESGGGVVQPGRSLRLSCAASGFTFSDYNMAWIRQAPGKGLEWVAAIIYDGTRTYYRDSVKGRFTISRDNSKSTLYLQMNSLRAEDTAVYYCATGDSYTNFAYWGQGTLVTVSSASTKGPSVFPLAPSSKSTSGGTAALGCLVKDYFPEPVTVSWNSGALTSGVHTFPAVLQSSGLYSLSSVVTVPSSSLGTQTYICNVNHKPSNTKVDKKVEPKSCDKTHTCPPCPAPELLGGPSVFLFPPKPKDTLMISRTPEVTCVVVDVSHEDPEVKFNWYVDGVEVHNAKTKPREEQYNSTYRVVSVLTVLHQDWLNGKEYKCKVSNKALPAPIEKTISKAKGQPREPQVYTLPPSRDELTKNQVSLTCLVKGFYPSDIAVEWESNGQPENNYKTTPPVLDSDGSFFLYSKLTVDKSRWQQGNVFSCSVMHEALHNHYTQKSLSLSPGK

SEQ ID NO: 60 - protein, 7 aa, synthetic construct
  source 1..7: note = Polypeptide
  SITE 5: note = X is Dap(Me2)
  SITE 7: note = X is Cit
GPRNXVX

SEQ ID NO: 61 - protein, 6 aa, synthetic construct
  source 1..6: note = Polypeptide
  SITE 6: note = X is Cit
PLSLVX

SEQ ID NO: 62 - protein, 9 aa, synthetic construct
  source 1..9: note = Polypeptide
GPRNLGGFG

SEQ ID NO: 63 - protein, 6 aa, synthetic construct
  source 1..6: note = Polypeptide
  SITE 2: note = X is Cit
  SITE 6: note = X is Cit
PXSLVX

SEQ ID NO: 64 - protein, 7 aa, synthetic construct
  source 1..7: note = Polypeptide
  SITE 3: note = X is Cit
  SITE 7: note = X is Cit
GPXNLVX

SEQ ID NO: 65 - protein, 7 aa, synthetic construct
  source 1..7: note = Polypeptide
  SITE 3: note = X is Cit
  SITE 5: note = X is Dap(Me2)
  SITE 7: note = X is Cit
SPXSXVX

SEQ ID NO: 66 - protein, 6 aa, synthetic construct
  source 1..6: note = Polypeptide
  SITE 4: note = X is Dap(Me2)
  SITE 6: note = X is Cit
PRSXVX

SEQ ID NO: 67 - protein, 6 aa, synthetic construct
  source 1..6: note = Polypeptide
  SITE 2: note = X is Cit
  SITE 6: note = X is Cit
PXNLVX

SEQ ID NO: 68 - protein, 6 aa, synthetic construct
  source 1..6: note = Polypeptide
  SITE 6: note = X is Cit
PASLVX